European Patent Application EP 4 681 729 A1, published January 21, 2026. Title: PHARMACEUTICAL COMPOSITION CONTAINING PD-1/PVRIG/TIGIT BINDING PROTEIN AND MEDICAL USE THEREOF. Applicant: SHANGHAI MABGEN BIOTECH LTD. The sequence listing filed with the application follows.

SEQUENCE LISTING (79 sequences)

SEQ ID NO: 1 - protein, 288 aa, Artificial Sequence
MQIPQAPWPVVWAVLQLGWRPGWFLDSPDRPWNPPTFSPALLVVTEGDNATFTCSFSNTSESFVLNWYRMSPSNQTDKLAAFPEDRSQPGQDCRFRVTQLPNGRDFHMSVVRARRNDSGTYLCGAISLAPKAQIKESLRAELRVTERRAEVPTAHPSPSPRPAGQFQTLVVGVVGGLLGSLVLLVWVLAVICSRAARGTIGARRTGQPLKEDPSAVPVFSVDYGELDFQWREKTPEPPVPCVPEQTEYATIVFPSGMGTSSPARRGSADGPRSAQPLRPEDGHCSWPL

SEQ ID NO: 2 - protein, 116 aa, Artificial Sequence
EVQVVESGGGLVQPGGSLRLSCVASGLTFSDYSMSWYRQAPGKERELVAIISGSGVIAHYVDSVKGRFTISRDNAKSTVYLQMVSLKPEDRGVYYCRAVSDWDDYWGQGTQVTVSS

SEQ ID NO: 3 - protein, 5 aa, Artificial Sequence
DYSMS

SEQ ID NO: 4 - protein, 17 aa, Artificial Sequence
IISGSGVIAHYVDSVKG

SEQ ID NO: 5 - protein, 7 aa, Artificial Sequence
VSDWDDY

SEQ ID NO: 6 - protein, 229 aa, Artificial Sequence
ESKYGPPCPPCPAPEFLGGPSVFLFPPKPKDTLMISRTPEVTCVVVDVSQEDPEVQFNWYVDGVEVHNAKTKPREEQFNSTYRVVSVLTVLHQDWLNGKEYKCKVSNKGLPSSIEKTISKAKGQPREPQVYTLPPSQEEMTKNQVSLTCLVKGFYPSDIAVEWESNGQPENNYKTTPPVLDSDGSFFLYSRLTVDKSRWQEGNVFSCSVMHEALHNHYTQKSLSLSLGK

SEQ ID NO: 7 - protein, 345 aa, Artificial Sequence
EVQVVESGGGLVQPGGSLRLSCVASGLTFSDYSMSWYRQAPGKERELVAIISGSGVIAHYVDSVKGRFTISRDNAKSTVYLQMVSLKPEDRGVYYCRAVSDWDDYWGQGTQVTVSSESKYGPPCPPCPAPEFLGGPSVFLFPPKPKDTLMISRTPEVTCVVVDVSQEDPEVQFNWYVDGVEVHNAKTKPREEQFNSTYRVVSVLTVLHQDWLNGKEYKCKVSNKGLPSSIEKTISKAKGQPREPQVYTLPPSQEEMTKNQVSLTCLVKGFYPSDIAVEWESNGQPENNYKTTPPVLDSDGSFFLYSRLTVDKSRWQEGNVFSCSVMHEALHNHYTQKSLSLSLGK

SEQ ID NO: 8 - protein, 116 aa, Artificial Sequence
EVQLQESGGGLVQPGGSLRLSCTASGLTFSDYSMSWYRQAPGKGRELVAIISGSGVIAHYVDSVKGRFTISRDNSKNTVYLQMRSLTPEDRAVYYCRAVSDWDDYWGQGTQVTVSS

SEQ ID NO: 9 - protein, 116 aa, Artificial Sequence
EVQLVESGGGLVQPGGSLRLSCAASGLTFSDYSMSWVRQAPGKGLEWVAIISGSGVIAHYVDSVKGRFTISRDNSKNTVYLQMNSLRAEDTAVYYCRAVSDWDDYWGQGTQVTVSS

SEQ ID NO: 10 - protein, 116 aa, Artificial Sequence
EVQLVESGGGLVQPGGSLRLSCAASGLTFSDYSMSWVRQAPGKGLEWVAIISGSGVIAHYVDSVKGRFTISRDNSKNTVYLQMNSLRAEDTAVYYCRAVSDWDEYWGQGTQVTVSS

SEQ ID NO: 11 - protein, 116 aa, Artificial Sequence
EVQLQESGGGLVQPGGSLRLSCTASGLTFSDYSMSWYRQAPGKGRELVAIISGSGVIAHYVDSVKGRFTISRDNAKNTVYLQMRSLTPEDRAVYYCRAVSDWDDYWGQGTQVTVSS

SEQ ID NO: 12 - protein, 116 aa, Artificial Sequence
EVQLQESGGGLVQPGGSLRLSCTASGLTFSDYSMSWYRQAPGKGRELVAIISGSGVITHYVDSVKGRFTISRDNSKNTVYLQMRSLTPEDRAVYYCRAVSDWDDYWGQGTQVTVSS

SEQ ID NO: 13 - protein, 116 aa, Artificial Sequence
EVQLQESGGGLVQPGGSLRLSCTASGLTFSDYSMSWYRQAPGKGRELVAIISGSGGIAHYVDSVKGRFTISRDNSKNTVYLQMRSLTPEDRAVYYCRAVSDWDDYWGQGTQVTVSS

SEQ ID NO: 14 - protein, 116 aa, Artificial Sequence
EVQLQESGGGLVQPGGSLRLSCTASGLTFSDYSMSWYRQAPGKGRELVAIISGSGVSAHYVDSVKGRFTISRDNSKNTVYLQMRSLTPEDRAVYYCRAVSDWDDYWGQGTQVTVSS

SEQ ID NO: 15 - protein, 116 aa, Artificial Sequence
EVQLQESGGGLVQPGGSLRLSCTASGLTFSDYSMSWYRQAPGKGRELVAIISGSGVIAHYVDSVKGRFTISRDNSKNTVYLQMRSLTPEDRAVYYCRAVSDWEDYWGQGTQVTVSS

SEQ ID NO: 16 - protein, 116 aa, Artificial Sequence
EVQLQESGGGLVQPGGSLRLSCTASGLTFSDYSMSWYRQAPGKGRELVAIISGSGVIAHYVDSVKGRFTISRDNSKNTVYLQMRSLTPEDRAVYYCRAVSDWDEYWGQGTQVTVSS

SEQ ID NO: 17 - protein, 116 aa, Artificial Sequence
EVQLQESGGGLVQPGGSLRLSCTASGLTFSDYSMSWYRQAPGKGRELVAIISGSGVIAHYVDSVKGRFTISRDNAKNTVYLQMRSLTPEDRAVYYCRAVSDWEDYWGQGTQVTVSS

SEQ ID NO: 18 - protein, 116 aa, Artificial Sequence
EVQLQESGGGLVQPGGSLRLSCTASGLTFSDYSMSWYRQAPGKGRELVAIISGSGVIAHYVDSVKGRFTISRDNAKNTVYLQMRSLTPEDRAVYYCRAVSDWDEYWGQGTQVTVSS

SEQ ID NO: 19 - protein, 116 aa, Artificial Sequence
EVQLQESGGGLVQPGGSLRLSCTASGLTFSDYSMSWYRQAPGKGRELVAIISGSGVITHYVDSVKGRFTISRDNAKNTVYLQMRSLTPEDRAVYYCRAVSDWEDYWGQGTQVTVSS

SEQ ID NO: 20 - protein, 116 aa, Artificial Sequence
EVQLQESGGGLVQPGGSLRLSCTASGLTFSDYSMSWYRQAPGKGRELVAIISGSGVITHYVDSVKGRFTISRDNAKNTVYLQMRSLTPEDRAVYYCRAVSDWDEYWGQGTQVTVSS

SEQ ID NO: 21 - protein, 116 aa, Artificial Sequence
EVQLQESGGGLVQPGGSLRLSCTASGLTFSDYSMSWYRQAPGKGRELVAIISGSGGIAHYVDSVKGRFTISRDNAKNTVYLQMRSLTPEDRAVYYCRAVSDWEDYWGQGTQVTVSS

SEQ ID NO: 22 - protein, 116 aa, Artificial Sequence
EVQLQESGGGLVQPGGSLRLSCTASGLTFSDYSMSWYRQAPGKGRELVAIISGSGGIAHYVDSVKGRFTISRDNAKNTVYLQMRSLTPEDRAVYYCRAVSDWDEYWGQGTQVTVSS

SEQ ID NO: 23 - protein, 116 aa, Artificial Sequence
EVQLQESGGGLVQPGGSLRLSCTASGLTFSDYSMSWYRQAPGKGRELVAIISGSGVSAHYVDSVKGRFTISRDNAKNTVYLQMRSLTPEDRAVYYCRAVSDWEDYWGQGTQVTVSS

SEQ ID NO: 24 - protein, 116 aa, Artificial Sequence
EVQLQESGGGLVQPGGSLRLSCTASGLTFSDYSMSWYRQAPGKGRELVAIISGSGVSAHYVDSVKGRFTISRDNAKNTVYLQMRSLTPEDRAVYYCRAVSDWDEYWGQGTQVTVSS

SEQ ID NO: 25 - protein, 116 aa, Artificial Sequence
EVQLQESGGGLVQPGGSLRLSCTASGLTFSDYSMSWYRQAPGKGRELVAIISGSGGITHYVDSVKGRFTISRDNAKNTVYLQMRSLTPEDRAVYYCRAVSDWEDYWGQGTQVTVSS

SEQ ID NO: 26 - protein, 116 aa, Artificial Sequence
EVQLVESGGGLVQPGGSLRLSCAASGFTFSDYSMSWYRQAPGKGRELVAIISGSGVITHYVDSVKGRFTISRDNAKNTLYLQMRSLRAEDTAVYYCRAVSDWEDYWGQGTQVTVSS

SEQ ID NO: 27 - protein, 116 aa, Artificial Sequence
EVQLVESGGGLVQPGGSLRLSCAASGLTFSDYSMSWYRQAPGKGRELVAIISGSGVITHYVDSVKGRFTISRDNAKNTLYLQMRSLRAEDTAVYYCRAVSDWEDYWGQGTQVTVSS

SEQ ID NO: 28 - protein, 116 aa, Artificial Sequence
EVQLVESGGGLVQPGGSLRLSCAASGLTFSDYSMSWYRQAPGKGRELVAIISGSGVITHYVDSVKGRFTISRDNAKNTVYLQMRSLRAEDTAVYYCRAVSDWEDYWGQGTQVTVSS

SEQ ID NO: 29 - protein, 116 aa, Artificial Sequence
EVQLVESGGGLVQPGGSLRLSCAASGLTFSDYSMSWYRQAPGKGRELVAIISGSGVITHYVDSVKGRFTISRDNAKNTVYLQMRSLRAEDRAVYYCRAVSDWEDYWGQGTQVTVSS

SEQ ID NO: 30 - protein, 17 aa, Artificial Sequence
  VARIANT 7: note; note (original language) = X is selected from the group consisting of V and G
  VARIANT 8: note; note (original language) = X is selected from the group consisting of I and S
  VARIANT 9: note; note (original language) = X is selected from the group consisting of T and A
IISGSGXXXHYVDSVKG

SEQ ID NO: 31 - protein, 7 aa, Artificial Sequence
  VARIANT 5: note; note (original language) = X is selected from the group consisting of D and E
  VARIANT 6: note; note (original language) = X is selected from the group consisting of D and E
VSDWXXY

SEQ ID NO: 32 - protein, 17 aa, Artificial Sequence
IISGSGVITHYVDSVKG

SEQ ID NO: 33 - protein, 17 aa, Artificial Sequence
IISGSGGIAHYVDSVKG

SEQ ID NO: 34 - protein, 17 aa, Artificial Sequence
IISGSGVSAHYVDSVKG

SEQ ID NO: 35 - protein, 7 aa, Artificial Sequence
VSDWEDY

SEQ ID NO: 36 - protein, 7 aa, Artificial Sequence
VSDWDEY

SEQ ID NO: 37 - protein, 137 aa, Artificial Sequence
TPEVWVQVQMEATELSSFTVHCGFLGPGSISLVTVSWGGPDGAGGTKLAVLHPELGTRQWAPARQARWETQSSISLALEDSGASSPFANTTFCCKFASFPEGSWESCGSLPPSSDPGLSAPPTPVPILRADHHHHHH

SEQ ID NO: 38 - protein, 127 aa, Artificial Sequence
HVQLVESGGGSVQAGGSLRLSCVASASGFTYRPYCMAWFRQAPGKEREAVAGIDIFGGTTYADSVKGRFTASRDNAGFSLFLQMNDLKPEDTAMYYCAAGDSPDGRCPPLGQGLNYWGQGTQVTVSS

SEQ ID NO: 39 - protein, 7 aa, Artificial Sequence
YRPYCMA

SEQ ID NO: 40 - protein, 16 aa, Artificial Sequence
GIDIFGGTTYADSVKG

SEQ ID NO: 41 - protein, 17 aa, Artificial Sequence
GDSPDGRCPPLGQGLNY

SEQ ID NO: 42 - protein, 229 aa, Artificial Sequence
ESKYGPPCPPCPAPEAAGGPSVFLFPPKPKDTLMISRTPEVTCVVVDVSQEDPEVQFNWYVDGVEVHNAKTKPREEQFNSTYRVVSVLTVLHQDWLNGKEYKCKVSNKGLPSSIEKTISKAKGQPREPQVYTLPPSQEEMTKNQVSLTCLVKGFYPSDIAVEWESNGQPENNYKTTPPVLDSDGSFFLYSRLTVDKSRWQEGNVFSCSVMHEALHNHYTQKSLSLSLGA

SEQ ID NO: 43 - protein, 356 aa, Artificial Sequence
HVQLVESGGGSVQAGGSLRLSCVASASGFTYRPYCMAWFRQAPGKEREAVAGIDIFGGTTYADSVKGRFTASRDNAGFSLFLQMNDLKPEDTAMYYCAAGDSPDGRCPPLGQGLNYWGQGTQVTVSSESKYGPPCPPCPAPEAAGGPSVFLFPPKPKDTLMISRTPEVTCVVVDVSQEDPEVQFNWYVDGVEVHNAKTKPREEQFNSTYRVVSVLTVLHQDWLNGKEYKCKVSNKGLPSSIEKTISKAKGQPREPQVYTLPPSQEEMTKNQVSLTCLVKGFYPSDIAVEWESNGQPENNYKTTPPVLDSDGSFFLYSRLTVDKSRWQEGNVFSCSVMHEALHNHYTQKSLSLSLGA

SEQ ID NO: 44 - protein, 449 aa, Artificial Sequence
EVQLVESGGGVVKPGGSLRLSCAASGFTFGTSSMNWVRQAPGKGLEWVAVISFDGTEIHYADSVKGRFTISRDNSKSTVFLQMNSLRPDDTALYYCAKGSGNIYFYSGMDVWGQGTTVTVSSASTKGPSVFPLAPCSRSTSESTAALGCLVKDYFPEPVTVSWNSGALTSGVHTFPAVLQSSGLYSLSSVVTVPSSSLGTKTYTCNVDHKPSNTKVDKRVESKYGPPCPPCPAPEAAGGPSVFLFPPKPKDTLMISRTPEVTCVVVDVSQEDPEVQFNWYVDGVEVHNAKTKPREEQFNSTYRVVSVLTVLHQDWLNGKEYKCKVSNKGLPSSIEKTISKAKGQPREPQVYTLPPSQEEMTKNQVSLTCLVKGFYPSDIAVEWESNGQPENNYKTTPPVLDSDGSFFLYSRLTVDKSRWQEGNVFSCSVMHEALHNHYTQKSLSLSLGA

SEQ ID NO: 45 - protein, 214 aa, Artificial Sequence
DIQMTQSPSTLSASVGDRVTITCRAGQSISGWLAWFQQKPGKAPNLLIYETSTLESGVPSRFSGSGSGTEYTLTISSLQPDDFATYYCQQYYSYPLTFGQGTKVEIKRTVAAPSVFIFPPSDEQLKSGTASVVCLLNNFYPREAKVQWKVDNALQSGNSQESVTEQDSKDSTYSLSSTLTLSKADYEKHKVYACEVTHQGLSSPVTKSFNRGEC

SEQ ID NO: 46 - protein, 125 aa, Artificial Sequence
EVQLVESGGGLVQPGGSLRLSCAASGFTYRPYCMAWFRQAPGKGLEAVAGIDIFGGTTYADSVKGRFTISRDNAKNSLYLQMNSLRAEDTAVYYCAAGDSPDGRCPPLGQGLNYWGQGTMVTVSS

SEQ ID NO: 47 - protein, 127 aa, Artificial Sequence
EVQLVESGGGLVQPGGSLRLSCVASASGFTYRPYCMAWFRQAPGKGLEAVAGIDIFGGTTYADSVKGRFTISRDNAKNSLYLQMNSLRAEDTAVYYCAAGDSPDGRCPPLGQGLNYWGQGTMVTVSS

SEQ ID NO: 48 - protein, 127 aa, Artificial Sequence
HVQLVESGGGLVQPGGSLRLSCVASASGFTYRPYCMAWFRQAPGKEREAVAGIDIFGGTTYADSVKGRFTASRDNAGFSLYLQMNSLRAEDTAVYYCAAGDSPDGRCPPLGQGLNYWGQGTMVTVSS

SEQ ID NO: 49 - protein, 127 aa, Artificial Sequence
EVQLVESGGGLVQPGGSLRLSCVASASGFTYRPYCMAWFRQAPGKGLEAVAGIDIFGGTTYADSVKGRFTISRDNAGFSLYLQMNSLRAEDTAVYYCAAGDSPDGRCPPLGQGLNYWGQGTMVTVSS

SEQ ID NO: 50 - protein, 127 aa, Artificial Sequence
HVQLVESGGGLVQPGGSLRLSCVASASGFTYRPYCMAWFRQAPGKGLEAVAGIDIFGGTTYADSVKGRFTASRDNAGFSLYLQMNSLRAEDTAVYYCAAGDSPDGRCPPLGQGLNYWGQGTMVTVSS

SEQ ID NO: 51 - protein, 446 aa, Artificial Sequence
EVQLVQSGAEVKKPGASVKVSCKASGYTFTNYWMHWVRQAPGQGLEWMGRIDPDSTGSKYNEKFKTRVTMTRDTSTSTVYMELSSLRSEDTAVYYCAREGAYGYYFDYWGQGTLVTVSSASTKGPSVFPLAPCSRSTSESTAALGCLVKDYFPEPVTVSWNSGALTSGVHTFPAVLQSSGLYSLSSVVTVPSSSLGTKTYTCNVDHKPSNTKVDKRVESKYGPPCPPCPAPEFLGGPSVFLFPPKPKDTLMISRTPEVTCVVVDVSQEDPEVQFNWYVDGVEVHNAKTKPREEQFNSTYRVVSVLTVLHQDWLNGKEYKCKVSNKGLPSSIEKTISKAKGQPREPQVYTLPPSQEEMTKNQVSLTCLVKGFYPSDIAVEWESNGQPENNYKTTPPVLDSDGSFFLYSRLTVDKSRWQEGNVFSCSVMHEALHNHYTQKSLSLSLGK

SEQ ID NO: 52 - protein, 214 aa, Artificial Sequence
DIQMTQSPSSLSASVGDRVTITCRASENIYSYLAWYQQKPGKSPKLLIYNARTLAEGVPSRFSGSGSGTDFTLTISSLQPEDFATYYCQYHSGSPLPFGGGTKVEIKRTVAAPSVFIFPPSDEQLKSGTASVVCLLNNFYPREAKVQWKVDNALQSGNSQESVTEQDSKDSTYSLSSTLTLSKADYEKHKVYACEVTHQGLSSPVTKSFNRGEC

SEQ ID NO: 53 - protein, 583 aa, Artificial Sequence
HVQLVESGGGSVQAGGSLRLSCVASASGFTYRPYCMAWFRQAPGKEREAVAGIDIFGGTTYADSVKGRFTASRDNAGFSLFLQMNDLKPEDTAMYYCAAGDSPDGRCPPLGQGLNYWGQGTQVTVSSGGGGSGGGGSEVQLVQSGAEVKKPGASVKVSCKASGYTFTNYWMHWVRQAPGQGLEWMGRIDPDSTGSKYNEKFKTRVTMTRDTSTSTVYMELSSLRSEDTAVYYCAREGAYGYYFDYWGQGTLVTVSSASTKGPSVFPLAPCSRSTSESTAALGCLVKDYFPEPVTVSWNSGALTSGVHTFPAVLQSSGLYSLSSVVTVPSSSLGTKTYTCNVDHKPSNTKVDKRVESKYGPPCPPCPAPEFLGGPSVFLFPPKPKDTLMISRTPEVTCVVVDVSQEDPEVQFNWYVDGVEVHNAKTKPREEQFNSTYRVVSVLTVLHQDWLNGKEYKCKVSNKGLPSSIEKTISKAKGQPREPQVYTLPPSQEEMTKNQVSLTCLVKGFYPSDIAVEWESNGQPENNYKTTPPVLDSDGSFFLYSRLTVDKSRWQEGNVFSCSVMHEALHNHYTQKSLSLSLGK

SEQ ID NO: 54 - protein, 583 aa, Artificial Sequence
EVQLVQSGAEVKKPGASVKVSCKASGYTFTNYWMHWVRQAPGQGLEWMGRIDPDSTGSKYNEKFKTRVTMTRDTSTSTVYMELSSLRSEDTAVYYCAREGAYGYYFDYWGQGTLVTVSSASTKGPSVFPLAPCSRSTSESTAALGCLVKDYFPEPVTVSWNSGALTSGVHTFPAVLQSSGLYSLSSVVTVPSSSLGTKTYTCNVDHKPSNTKVDKRVESKYGPPCPPCPAPEFLGGPSVFLFPPKPKDTLMISRTPEVTCVVVDVSQEDPEVQFNWYVDGVEVHNAKTKPREEQFNSTYRVVSVLTVLHQDWLNGKEYKCKVSNKGLPSSIEKTISKAKGQPREPQVYTLPPSQEEMTKNQVSLTCLVKGFYPSDIAVEWESNGQPENNYKTTPPVLDSDGSFFLYSRLTVDKSRWQEGNVFSCSVMHEALHNHYTQKSLSLSLGKGGGGSGGGGSHVQLVESGGGSVQAGGSLRLSCVASASGFTYRPYCMAWFRQAPGKEREAVAGIDIFGGTTYADSVKGRFTASRDNAGFSLFLQMNDLKPEDTAMYYCAAGDSPDGRCPPLGQGLNYWGQGTQVTVSS

SEQ ID NO: 55 - protein, 351 aa, Artificial Sequence
HVQLVESGGGSVQAGGSLRLSCVASASGFTYRPYCMAWFRQAPGKEREAVAGIDIFGGTTYADSVKGRFTASRDNAGFSLFLQMNDLKPEDTAMYYCAAGDSPDGRCPPLGQGLNYWGQGTQVTVSSGGGGSGGGGSDIQMTQSPSSLSASVGDRVTITCRASENIYSYLAWYQQKPGKSPKLLIYNARTLAEGVPSRFSGSGSGTDFTLTISSLQPEDFATYYCQYHSGSPLPFGGGTKVEIKRTVAAPSVFIFPPSDEQLKSGTASVVCLLNNFYPREAKVQWKVDNALQSGNSQESVTEQDSKDSTYSLSSTLTLSKADYEKHKVYACEVTHQGLSSPVTKSFNRGEC

SEQ ID NO: 56 - protein, 351 aa, Artificial Sequence
DIQMTQSPSSLSASVGDRVTITCRASENIYSYLAWYQQKPGKSPKLLIYNARTLAEGVPSRFSGSGSGTDFTLTISSLQPEDFATYYCQYHSGSPLPFGGGTKVEIKRTVAAPSVFIFPPSDEQLKSGTASVVCLLNNFYPREAKVQWKVDNALQSGNSQESVTEQDSKDSTYSLSSTLTLSKADYEKHKVYACEVTHQGLSSPVTKSFNRGECGGGGSGGGGSHVQLVESGGGSVQAGGSLRLSCVASASGFTYRPYCMAWFRQAPGKEREAVAGIDIFGGTTYADSVKGRFTASRDNAGFSLFLQMNDLKPEDTAMYYCAAGDSPDGRCPPLGQGLNYWGQGTQVTVSS

SEQ ID NO: 57 - protein, 5 aa, Artificial Sequence
NYWMH

SEQ ID NO: 58 - protein, 17 aa, Artificial Sequence
RIDPDSTGSKYNEKFKT

SEQ ID NO: 59 - protein, 10 aa, Artificial Sequence
EGAYGYYFDY

SEQ ID NO: 60 - protein, 11 aa, Artificial Sequence
RASENIYSYLA

SEQ ID NO: 61 - protein, 7 aa, Artificial Sequence
NARTLAE

SEQ ID NO: 62 - protein, 9 aa, Artificial Sequence
QYHSGSPLP

SEQ ID NO: 63 - protein, 119 aa, Artificial Sequence
EVQLVQSGAEVKKPGASVKVSCKASGYTFTNYWMHWVRQAPGQGLEWMGRIDPDSTGSKYNEKFKTRVTMTRDTSTSTVYMELSSLRSEDTAVYYCAREGAYGYYFDYWGQGTLVTVSS

SEQ ID NO: 64 - protein, 119 aa, Artificial Sequence
EVQLVQSGAEVKKPGASVKVSCKASGYTFTNYWMHWVRQAPGQGLEWMGRIDPDSTGSKYNEKFKTRVTMTVDTSTSTVYMELSSLRSEDTAVYYCAREGAYGYYFDYWGQGTLVTVSS

SEQ ID NO: 65 - protein, 119 aa, Artificial Sequence
EVQLVQSGAEVKKPGASVKVSCKASGYTFTNYWMHWVRQAPGQGLEWIGRIDPDSTGSKYNEKFKTRVTMTVDTSTSTAYMELSSLRSEDTAVYYCAREGAYGYYFDYWGQGTLVTVSS

SEQ ID NO: 66 - protein, 107 aa, Artificial Sequence
DIQMTQSPSSLSASVGDRVTITCRASENIYSYLAWYQQKPGKAPKLLIYNARTLAEGVPSRFSGSGSGTDFTLTISSLQPEDFATYYCQYHSGSPLPFGGGTKVEIK

SEQ ID NO: 67 - protein, 107 aa, Artificial Sequence
DIQMTQSPSSLSASVGDRVTITCRASENIYSYLAWYQQKPGKSPKLLIYNARTLAEGVPSRFSGSGSGTDFTLTISSLQPEDFATYYCQYHSGSPLPFGGGTKVEIK

SEQ ID NO: 68 - protein, 583 aa, Artificial Sequence
HVQLVESGGGLVQPGGSLRLSCVASASGFTYRPYCMAWFRQAPGKEREAVAGIDIFGGTTYADSVKGRFTASRDNAGFSLYLQMNSLRAEDTAVYYCAAGDSPDGRCPPLGQGLNYWGQGTMVTVSSGGGGSGGGGSEVQLVQSGAEVKKPGASVKVSCKASGYTFTNYWMHWVRQAPGQGLEWMGRIDPDSTGSKYNEKFKTRVTMTRDTSTSTVYMELSSLRSEDTAVYYCAREGAYGYYFDYWGQGTLVTVSSASTKGPSVFPLAPCSRSTSESTAALGCLVKDYFPEPVTVSWNSGALTSGVHTFPAVLQSSGLYSLSSVVTVPSSSLGTKTYTCNVDHKPSNTKVDKRVESKYGPPCPPCPAPEFLGGPSVFLFPPKPKDTLMISRTPEVTCVVVDVSQEDPEVQFNWYVDGVEVHNAKTKPREEQFNSTYRVVSVLTVLHQDWLNGKEYKCKVSNKGLPSSIEKTISKAKGQPREPQVYTLPPSQEEMTKNQVSLTCLVKGFYPSDIAVEWESNGQPENNYKTTPPVLDSDGSFFLYSRLTVDKSRWQEGNVFSCSVMHEALHNHYTQKSLSLSLGK

SEQ ID NO: 69 - protein, 583 aa, Artificial Sequence
EVQLVESGGGLVQPGGSLRLSCVASASGFTYRPYCMAWFRQAPGKGLEAVAGIDIFGGTTYADSVKGRFTISRDNAGFSLYLQMNSLRAEDTAVYYCAAGDSPDGRCPPLGQGLNYWGQGTMVTVSSGGGGSGGGGSEVQLVQSGAEVKKPGASVKVSCKASGYTFTNYWMHWVRQAPGQGLEWMGRIDPDSTGSKYNEKFKTRVTMTRDTSTSTVYMELSSLRSEDTAVYYCAREGAYGYYFDYWGQGTLVTVSSASTKGPSVFPLAPCSRSTSESTAALGCLVKDYFPEPVTVSWNSGALTSGVHTFPAVLQSSGLYSLSSVVTVPSSSLGTKTYTCNVDHKPSNTKVDKRVESKYGPPCPPCPAPEFLGGPSVFLFPPKPKDTLMISRTPEVTCVVVDVSQEDPEVQFNWYVDGVEVHNAKTKPREEQFNSTYRVVSVLTVLHQDWLNGKEYKCKVSNKGLPSSIEKTISKAKGQPREPQVYTLPPSQEEMTKNQVSLTCLVKGFYPSDIAVEWESNGQPENNYKTTPPVLDSDGSFFLYSRLTVDKSRWQEGNVFSCSVMHEALHNHYTQKSLSLSLGK

SEQ ID NO: 70 - protein, 709 aa, Artificial Sequence
EVQLVESGGGLVQPGGSLRLSCAASGLTFSDYSMSWYRQAPGKGRELVAIISGSGVITHYVDSVKGRFTISRDNAKNTLYLQMRSLRAEDTAVYYCRAVSDWEDYWGQGTQVTVSSGGGGSGGGGSHVQLVESGGGLVQPGGSLRLSCVASASGFTYRPYCMAWFRQAPGKEREAVAGIDIFGGTTYADSVKGRFTASRDNAGFSLYLQMNSLRAEDTAVYYCAAGDSPDGRCPPLGQGLNYWGQGTMVTVSSGGGGSGGGGSEVQLVQSGAEVKKPGASVKVSCKASGYTFTNYWMHWVRQAPGQGLEWMGRIDPDSTGSKYNEKFKTRVTMTRDTSTSTVYMELSSLRSEDTAVYYCAREGAYGYYFDYWGQGTLVTVSSASTKGPSVFPLAPCSRSTSESTAALGCLVKDYFPEPVTVSWNSGALTSGVHTFPAVLQSSGLYSLSSVVTVPSSSLGTKTYTCNVDHKPSNTKVDKRVESKYGPPCPPCPAPEFLGGPSVFLFPPKPKDTLMISRTPEVTCVVVDVSQEDPEVQFNWYVDGVEVHNAKTKPREEQFNSTYRVVSVLTVLHQDWLNGKEYKCKVSNKGLPSSIEKTISKAKGQPREPQVYTLPPSQEEMTKNQVSLTCLVKGFYPSDIAVEWESNGQPENNYKTTPPVLDSDGSFFLYSRLTVDKSRWQEGNVFSCSVMHEALHNHYTQKSLSLSLGK

SEQ ID NO: 71 - protein, 340 aa, Artificial Sequence
EVQLVESGGGLVQPGGSLRLSCAASGLTFSDYSMSWYRQAPGKGRELVAIISGSGVITHYVDSVKGRFTISRDNAKNTLYLQMRSLRAEDTAVYYCRAVSDWEDYWGQGTQVTVSSGGGGSGGGGSDIQMTQSPSSLSASVGDRVTITCRASENIYSYLAWYQQKPGKSPKLLIYNARTLAEGVPSRFSGSGSGTDFTLTISSLQPEDFATYYCQYHSGSPLPFGGGTKVEIKRTVAAPSVFIFPPSDEQLKSGTASVVCLLNNFYPREAKVQWKVDNALQSGNSQESVTEQDSKDSTYSLSSTLTLSKADYEKHKVYACEVTHQGLSSPVTKSFNRGEC

SEQ ID NO: 72 - protein, 709 aa, Artificial Sequence
HVQLVESGGGLVQPGGSLRLSCVASASGFTYRPYCMAWFRQAPGKEREAVAGIDIFGGTTYADSVKGRFTASRDNAGFSLYLQMNSLRAEDTAVYYCAAGDSPDGRCPPLGQGLNYWGQGTMVTVSSGGGGSGGGGSEVQLVQSGAEVKKPGASVKVSCKASGYTFTNYWMHWVRQAPGQGLEWMGRIDPDSTGSKYNEKFKTRVTMTRDTSTSTVYMELSSLRSEDTAVYYCAREGAYGYYFDYWGQGTLVTVSSASTKGPSVFPLAPCSRSTSESTAALGCLVKDYFPEPVTVSWNSGALTSGVHTFPAVLQSSGLYSLSSVVTVPSSSLGTKTYTCNVDHKPSNTKVDKRVESKYGPPCPPCPAPEFLGGPSVFLFPPKPKDTLMISRTPEVTCVVVDVSQEDPEVQFNWYVDGVEVHNAKTKPREEQFNSTYRVVSVLTVLHQDWLNGKEYKCKVSNKGLPSSIEKTISKAKGQPREPQVYTLPPSQEEMTKNQVSLTCLVKGFYPSDIAVEWESNGQPENNYKTTPPVLDSDGSFFLYSRLTVDKSRWQEGNVFSCSVMHEALHNHYTQKSLSLSLGKGGGGSGGGGSEVQLVESGGGLVQPGGSLRLSCAASGLTFSDYSMSWYRQAPGKGRELVAIISGSGVITHYVDSVKGRFTISRDNAKNTLYLQMRSLRAEDTAVYYCRAVSDWEDYWGQGTQVTVSS

SEQ ID NO: 73 - protein, 340 aa, Artificial Sequence
DIQMTQSPSSLSASVGDRVTITCRASENIYSYLAWYQQKPGKSPKLLIYNARTLAEGVPSRFSGSGSGTDFTLTISSLQPEDFATYYCQYHSGSPLPFGGGTKVEIKRTVAAPSVFIFPPSDEQLKSGTASVVCLLNNFYPREAKVQWKVDNALQSGNSQESVTEQDSKDSTYSLSSTLTLSKADYEKHKVYACEVTHQGLSSPVTKSFNRGECGGGGSGGGGSEVQLVESGGGLVQPGGSLRLSCAASGLTFSDYSMSWYRQAPGKGRELVAIISGSGVITHYVDSVKGRFTISRDNAKNTLYLQMRSLRAEDTAVYYCRAVSDWEDYWGQGTQVTVSS

SEQ ID NO: 74 - protein, 127 aa, Artificial Sequence
EVQLVESGGGLVQPGGSLRLSCVASASGFTYRPYCMAWFRQAPGKEREAVAGIDIFGGTTYADSVKGRFTASRDNAGFSLYLQMNSLRAEDTAVYYCAAGDSPDGRCPPLGQGLNYWGQGTMVTVSS

SEQ ID NO: 75 - protein, 127 aa, Artificial Sequence
QVQLVESGGGLVQPGGSLRLSCVASASGFTYRPYCMAWFRQAPGKEREAVAGIDIFGGTTYADSVKGRFTASRDNAGFSLYLQMNSLRAEDTAVYYCAAGDSPDGRCPPLGQGLNYWGQGTMVTVSS

SEQ ID NO: 76 - protein, 709 aa, Artificial Sequence
EVQLVESGGGLVQPGGSLRLSCVASASGFTYRPYCMAWFRQAPGKEREAVAGIDIFGGTTYADSVKGRFTASRDNAGFSLYLQMNSLRAEDTAVYYCAAGDSPDGRCPPLGQGLNYWGQGTMVTVSSGGGGSGGGGSEVQLVQSGAEVKKPGASVKVSCKASGYTFTNYWMHWVRQAPGQGLEWMGRIDPDSTGSKYNEKFKTRVTMTRDTSTSTVYMELSSLRSEDTAVYYCAREGAYGYYFDYWGQGTLVTVSSASTKGPSVFPLAPCSRSTSESTAALGCLVKDYFPEPVTVSWNSGALTSGVHTFPAVLQSSGLYSLSSVVTVPSSSLGTKTYTCNVDHKPSNTKVDKRVESKYGPPCPPCPAPEFLGGPSVFLFPPKPKDTLMISRTPEVTCVVVDVSQEDPEVQFNWYVDGVEVHNAKTKPREEQFNSTYRVVSVLTVLHQDWLNGKEYKCKVSNKGLPSSIEKTISKAKGQPREPQVYTLPPSQEEMTKNQVSLTCLVKGFYPSDIAVEWESNGQPENNYKTTPPVLDSDGSFFLYSRLTVDKSRWQEGNVFSCSVMHEALHNHYTQKSLSLSLGKGGGGSGGGGSEVQLVESGGGLVQPGGSLRLSCAASGLTFSDYSMSWYRQAPGKGRELVAIISGSGVITHYVDSVKGRFTISRDNAKNTLYLQMRSLRAEDTAVYYCRAVSDWEDYWGQGTQVTVSS

SEQ ID NO: 77 - protein, 709 aa, Artificial Sequence
QVQLVESGGGLVQPGGSLRLSCVASASGFTYRPYCMAWFRQAPGKEREAVAGIDIFGGTTYADSVKGRFTASRDNAGFSLYLQMNSLRAEDTAVYYCAAGDSPDGRCPPLGQGLNYWGQGTMVTVSSGGGGSGGGGSEVQLVQSGAEVKKPGASVKVSCKASGYTFTNYWMHWVRQAPGQGLEWMGRIDPDSTGSKYNEKFKTRVTMTRDTSTSTVYMELSSLRSEDTAVYYCAREGAYGYYFDYWGQGTLVTVSSASTKGPSVFPLAPCSRSTSESTAALGCLVKDYFPEPVTVSWNSGALTSGVHTFPAVLQSSGLYSLSSVVTVPSSSLGTKTYTCNVDHKPSNTKVDKRVESKYGPPCPPCPAPEFLGGPSVFLFPPKPKDTLMISRTPEVTCVVVDVSQEDPEVQFNWYVDGVEVHNAKTKPREEQFNSTYRVVSVLTVLHQDWLNGKEYKCKVSNKGLPSSIEKTISKAKGQPREPQVYTLPPSQEEMTKNQVSLTCLVKGFYPSDIAVEWESNGQPENNYKTTPPVLDSDGSFFLYSRLTVDKSRWQEGNVFSCSVMHEALHNHYTQKSLSLSLGKGGGGSGGGGSEVQLVESGGGLVQPGGSLRLSCAASGLTFSDYSMSWYRQAPGKGRELVAIISGSGVITHYVDSVKGRFTISRDNAKNTLYLQMRSLRAEDTAVYYCRAVSDWEDYWGQGTQVTVSS

SEQ ID NO: 78 - protein, 10 aa, Artificial Sequence
GGGGSGGGGS

SEQ ID NO: 79 - protein, 17 aa, Artificial Sequence
IISGSGGITHYVDSVKG